European Patent Application EP 4 692 357 A1, published February 11, 2026. Title: Isocitrate Lyase and Use Thereof In Preparation of L-amino Acid. Applicant: Ningxia EPPEN Biotech Co., Ltd. Application CN. The sequence listing filed with the application follows.

SEQUENCE LISTING (36 sequences)

SEQ ID NO: 1 - DNA, 1305 bp, synthetic construct
  source 1..1305: mol_type = other DNA
atgaaaacccgtacacaacaaattgaagaattacagaaagagtggactcaaccgcgttgggaaggcattactcgcccatacagtgcggaagatgtggtgaaattacgcggttcagtcaatcctgaatgcacgctggcgcaactgggcgcagcgaaaatgtggcgtctgctgcacggtgagtcgaaaaaaggctacatcaacagcctcggcgcactgactggcggtcaggcgctgcaacaggcgaaagcgggtattgaagcagtctatctgtcgggatggcaggtagcggcggacgctaacctggcggccagcatgtatccggatcagtcgctctatccggcaaactcggtgccagctgtggtggagcggatcaacaacaccttccgtcgtgccgatcagatccaatggtccgcgggcattgagccgggcgatccgcgctatgtcgattacttcctgccgatcgttgccgatgcggaagccggttttggcggtgtcctgaatgcctttgaactgatgaaagcgatgattgaagccggtgcagcggcagttcacttcgaagatcagctggcgtcagtgaagaaatgcggtcacatgggcggcaaagttttagtgccaactcaggaagctattcagaaactggtcgcggcgcgtctggcagctgacgtgacgggcgttccaaccctgctggttgcccgtaccgatgctgatgcggcggatctgatcacctccgattgcgacccgtatgacagcgaatttattaccggcgagcgtaccagtgaaggcttcttccgtactcatgcgggcattgagcaagcgatcagccgtggcctggcgtatgcgccatatgctgacctggtctggtgtgaaacctccacgccggatctggaactggcgcgtcgctttgcacaagctatccacgcgaaatatccgggcaaactgctggcttataactgctcgccgtcgttcaactggcagaaaaacctcgacgacaaaactattgccagcttccagcagcagctgtcggatatgggctacaagttccagttcatcaccctggcaggtatccacagcatgtggttcaacatgtttgacctggcaaacgcctatgcccagggcgagggtatgaagcactacgttgagaaagtgcagcagccggaatttgccgccgcgaaagatggctataccttcgtatctcaccagcaggaagtgggtacaggttacttcgataaagtgacgactattattcagggcggcacgtcttcagtcaccgcgctgaccggctccactgaagaatcgcagttctaa

SEQ ID NO: 2 - protein, 434 aa, Escherichia coli
MKTRTQQIEELQKEWTQPRWEGITRPYSAEDVVKLRGSVNPECTLAQLGAAKMWRLLHGESKKGYINSLGALTGGQALQQAKAGIEAVYLSGWQVAADANLAASMYPDQSLYPANSVPAVVERINNTFRRADQIQWSAGIEPGDPRYVDYFLPIVADAEAGFGGVLNAFELMKAMIEAGAAAVHFEDQLASVKKCGHMGGKVLVPTQEAIQKLVAARLAADVTGVPTLLVARTDADAADLITSDCDPYDSEFITGERTSEGFFRTHAGIEQAISRGLAYAPYADLVWCETSTPDLELARRFAQAIHAKYPGKLLAYNCSPSFNWQKNLDDKTIASFQQQLSDMGYKFQFITLAGIHSMWFNMFDLANAYAQGEGMKHYVEKVQQPEFAAAKDGYTFVSHQQEVGTGYFDKVTTIIQGGTSSVTALTGSTEESQF

SEQ ID NO: 3 - DNA, 1602 bp, synthetic construct
  source 1..1602: mol_type = other DNA
tcttctgtgatagtcgatcgttaagcgattcagcaccttacctcaggcaccttcgggtgccttttttatttccgaaacgtacctcagcaggtgaataaattttattcatattgttatcaacaagttatcaagtatttttaattaaaatggaaattgtttttgattttgcattttaaatgagtagtcttagttgtgctgaacgaaaagagcacaacgatccttcgttcacagtggggaagttttcggatccatgacgaggagctgcacgaccaccacataactatggagcatctgcacatgaaaacccgtacacaacaaattgaagaattacagaaagagtggactcaaccgcgttgggaaggcattactcgcccatacagtgcggaagatgtggtgaaattacgcggttcagtcaatcctgaatgcacgctggcgcaactgggcgcagcgaaaatgtggcgtctgctgcacggtgagtcgaaaaaaggctacatcaacagcctcggcgcactgactggcggtcaggcgctgcaacaggcgaaagcgggtattgaagcagtctatctgtcgggatggcaggtagcggcggacgctaacctggcggccagcatgtatccggatcagtcgctctatccggcaaactcggtgccagctgtggtggagcggatcaacaacaccttccgtcgtgccgatcagatccaatggtccgcgggcattgagccgggcgatccgcgctatgtcgattacttcctgccgatcgttgccgatgcggaagccggttttggcggtgtcctgaatgcctttgaactgatgaaagcgatgattgaagccggtgcagcggcagttcacttcgaagatcagctggcgtcagtgaagaaatgcggtcacatgggcggcaaagttttagtgccaactcaggaagctattcagaaactggtcgcggcgcgtctggcagctgacgtgacgggcgttccaaccctgctggttgcccgtaccgatgctgatgcggcggatctgatcacctccgattgcgacccgtatgacagcgaatttattaccggcgagcgtaccagtgaaggcttcttccgtactcatgcgggcattgagcaagcgatcagccgtggcctggcgtatgcgccatatgctgacctggtctggtgtgaaacctccacgccggatctggaactggcgcgtcgctttgcacaagctatccacgcgaaatatccgggcaaactgctggcttataactgctcgccgtcgttcaactggcagaaaaacctcgacgacaaaactattgccagcttccagcagcagctgtcggatatgggctacaagttccagttcatcaccctggcaggtatccacagcatgtggttcaacatgtttgacctggcaaacgcctatgcccagggcgagggtatgaagcactacgttgagaaagtgcagcagccggaatttgccgccgcgaaagatggctataccttcgtatctcaccagcaggaagtgggtacaggttacttcgataaagtgacgactattattcagggcggcacgtcttcagtcaccgcgctgaccggctccactgaagaatcgcagttctaa

SEQ ID NO: 4 - DNA, 1889 bp, synthetic construct
  source 1..1889: mol_type = other DNA
taatacgactcactataggggaattgtgagcggataacaattcccctctagaaataattttgtttaactttaagaaggagatataccatgggcagcagccatcatcatcatcatcacagcagcggcctggtgccgcgcggcagccatatggctagcatgactggtggacagcaaatgggtcgcggatcctcttctgtgatagtcgatcgttaagcgattcagcaccttacctcaggcaccttcgggtgccttttttatttccgaaacgtacctcagcaggtgaataaattttattcatattgttatcaacaagttatcaagtatttttaattaaaatggaaattgtttttgattttgcattttaaatgagtagtcttagttgtgctgaacgaaaagagcacaacgatccttcgttcacagtggggaagttttcggatccatgacgaggagctgcacgaccaccacataactatggagcatctgcacatgaaaacccgtacacaacaaattgaagaattacagaaagagtggactcaaccgcgttgggaaggcattactcgcccatacagtgcggaagatgtggtgaaattacgcggttcagtcaatcctgaatgcacgctggcgcaactgggcgcagcgaaaatgtggcgtctgctgcacggtgagtcgaaaaaaggctacatcaacagcctcggcgcactgactggcggtcaggcgctgcaacaggcgaaagcgggtattgaagcagtctatctgtcgggatggcaggtagcggcggacgctaacctggcggccagcatgtatccggatcagtcgctctatccggcaaactcggtgccagctgtggtggagcggatcaacaacaccttccgtcgtgccgatcagatccaatggtccgcgggcattgagccgggcgatccgcgctatgtcgattacttcctgccgatcgttgccgatgcggaagccggttttggcggtgtcctgaatgcctttgaactgatgaaagcgatgattgaagccggtgcagcggcagttcacttcgaagatcagctggcgtcagtgaagaaatgcggtcacatgggcggcaaagttttagtgccaactcaggaagctattcagaaactggtcgcggcgcgtctggcagctgacgtgacgggcgttccaaccctgctggttgcccgtaccgatgctgatgcggcggatctgatcacctccgattgcgacccgtatgacagcgaatttattaccggcgagcgtaccagtgaaggcttcttccgtactcatgcgggcattgagcaagcgatcagccgtggcctggcgtatgcgccatatgctgacctggtctggtgtgaaacctccacgccggatctggaactggcgcgtcgctttgcacaagctatccacgcgaaatatccgggcaaactgctggcttataactgctcgccgtcgttcaactggcagaaaaacctcgacgacaaaactattgccagcttccagcagcagctgtcggatatgggctacaagttccagttcatcaccctggcaggtatccacagcatgtggttcaacatgtttgacctggcaaacgcctatgcccagggcgagggtatgaagcactacgttgagaaagtgcagcagccggaatttgccgccgcgaaagatggctataccttcgtatctcaccagcaggaagtgggtacaggttacttcgataaagtgacgactattattcagggcggcacgtcttcagtcaccgcgctgaccggctccactgaagaatcgcagttctaagcactcgagcaccaccaccaccaccactgagatccggctgctaacaaagcccgaaaggaagctgagttggctgctgccaccgctgagcaataactagc

SEQ ID NO: 5 - DNA, 1305 bp, synthetic construct
  source 1..1305: mol_type = other DNA
atgaaaacccgtacacaacaaattgaagaattacagaaagagtggactcaaccgcgttgggaaggcattactcgcccatacagtgcggaagatgtggtgaaattacgcggttcagtcaatcctgaatgcacgctggcgcaactgggcgcagcgaaaatgtggcgtctgctgcacggtgagtcgaaaaaaggctacatcaacagcctcggcgcactgactggcggtcaggcgctgcaacaggcgaaagcgggtattgaagcagtctatctgtcgggatggcaggtagcggcggacgctaacctggcggccagcatgtatccggatcagtcgctctatccggcaaactcggtgccagctgtggtggagcggatcaacaacaccttccgtcgtgccgatcagatccaatggtccgcgggcattgagccgggcgatccgcgctatgtcgattacttcctgccgatcgttgccgatgcggaagccggttttggcggtgtcctgaatgcctttgaactgatgaaagcgatgattgaagccggtgcagcggcagttcacttcgaagatcagctggcgtcagtgaagaaatgcggtcacatgggcggcaaagttttagtgccaactcaggaagctattcagaaactggtcgcggcgcgtctggcagctgacgtgacgggcgttccaaccctgctggttgcccgtaccgatgctgatgcggcggatctgatcacctccgattgcgacccgtatgacagcgaatttattaccggcgagcgtaccagtgaaggcttcttccgtactcatgcgggcattgagcaagcgatcagccgtggcctggcgtatgcgccatatgctgacctggtctggtgtgaaacctccacgccggatctggaactggcgcgtcgctttgcacaagctatccacgcgaaatatccgggcaaactgctggcttataactgctcgccgtcgttcaactggcagaaaaacctcgacgacaaaactattgccagcttccagcagcagctgtcggatatgggctacaagttccagttcatcaccctggcaggtatccacagcatgtggttcaacatgtttgacctggcaaacgcctatgcctagggcgagggtatgaagcactacgttgagaaagtgcagcagccggaatttgccgccgcgaaagatggctataccttcgtatctcaccagcaggaagtgggtacaggttacttcgataaagtgacgactattattcagggcggcacgtcttcagtcaccgcgctgaccggctccactgaagaatcgcagttctaa

SEQ ID NO: 6 - protein, 370 aa, synthetic construct
MKTRTQQIEELQKEWTQPRWEGITRPYSAEDVVKLRGSVNPECTLAQLGAAKMWRLLHGESKKGYINSLGALTGGQALQQAKAGIEAVYLSGWQVAADANLAASMYPDQSLYPANSVPAVVERINNTFRRADQIQWSAGIEPGDPRYVDYFLPIVADAEAGFGGVLNAFELMKAMIEAGAAAVHFEDQLASVKKCGHMGGKVLVPTQEAIQKLVAARLAADVTGVPTLLVARTDADAADLITSDCDPYDSEFITGERTSEGFFRTHAGIEQAISRGLAYAPYADLVWCETSTPDLELARRFAQAIHAKYPGKLLAYNCSPSFNWQKNLDDKTIASFQQQLSDMGYKFQFITLAGIHSMWFNMFDLANAYA

SEQ ID NO: 7 - DNA, 1241 bp, synthetic construct
  source 1..1241: mol_type = other DNA
ttggcggtgtcctgaatgcctttgaactgatgaaagcgatgattgaagccggtgcagcggcagttcacttcgaagatcagctggcgtcagtgaagaaatgcggtcacatgggcggcaaagttttagtgccaactcaggaagctattcagaaactggtcgcggcgcgtctggcagctgacgtgacgggcgttccaaccctgctggttgcccgtaccgatgctgatgcggcggatctgatcacctccgattgcgacccgtatgacagcgaatttattaccggcgagcgtaccagtgaaggcttcttccgtactcatgcgggcattgagcaagcgatcagccgtggcctggcgtatgcgccatatgctgacctggtctggtgtgaaacctccacgccggatctggaactggcgcgtcgctttgcacaagctatccacgcgaaatatccgggcaaactgctggcttataactgctcgccgtcgttcaactggcagaaaaacctcgacgacaaaactattgccagcttccagcagcagctgtcggatatgggctacaagttccagttcatcaccctggcaggtatccacagcatgtggttcaacatgtttgacctggcaaacgcctatgcctagggcgagggtatgaagcactacgttgagaaagtgcagcagccggaatttgccgccgcgaaagatggctataccttcgtatctcaccagcaggaagtgggtacaggttacttcgataaagtgacgactattattcagggcggcacgtcttcagtcaccgcgctgaccggctccactgaagaatcgcagttctaagcaacaacaaccgttgctgactgtaggccggataaggcgttcacgccgcatccggcaatcggtgcacgatgcctgatgcgacgcttgcgcgtcttatcatgcctacagccgttgccgaacgtaggctggataaggcgtttacgccgcatccggcaattctctgctcctgatgagggcgctaaatgccgcgtggcctggaattattgattgctcaaaccattttgcaaggcttcgatgctcagtatggtcgattcctcgaagtgacctccggtgcgcagcagcgtttcgaacaggccgactggcatgctgtccagcaggcgatgaaaaaccgtatccatctttacgatcatcacgttggtctggtcgtggagcaactgcgctgcattactaacggccaaagtacggacgcggcatttttac

SEQ ID NO: 8 - DNA, 943 bp, synthetic construct
  source 1..943: mol_type = other DNA
gcagtggcggttttcatggcttgttatgactgtttttttggggtacagtctatgcctcgggcatccaagcagcaagcgcgttacgccgtgggtcgatgtttgatgttatggagcagcaacgatgttacgcagcagggcagtcgccctaaaacaaagttaaacatcatgagggaagcggtgatcgccgaagtatcgactcaactatcagaggtagttggcgtcatcgagcgccatctcgaaccgacgttgctggccgtacatttgtacggctccgcagtggatggcggcctgaagccacacagtgatattgatttgctggttacggtgaccgtaaggcttgatgaaacaacgcggcgagctttgatcaacgaccttttggaaacttcggcttcccctggagagagcgagattctccgcgctgtagaagtcaccattgttgtgcacgacgacatcattccgtggcgttatccagctaagcgcgaactgcaatttggagaatggcagcgcaatgacattcttgcaggtatcttcgagccagccacgatcgacattgatctggctatcttgctgacaaaagcaagagaacatagcgttgccttggtaggtccagcggcggaggaactctttgatccggttcctgaacaggatctatttgaggcgctaaatgaaaccttaacgctatggaactcgccgcccgactgggctggcgatgagcgaaatgtagtgcttacgttgtcccgcatttggtacagcgcagtaaccggcaaaatcgcgccgaaggatgtcgctgccgactgggcaatggagcgcctgccggcccagtatcagcccgtcatacttgaagctagacaggcttatcttggacaagaagaagatcgcttggcctcgcgcgcagatcagttggaagaatttgtccactacgtgaaaggcgagatcaccaagg

SEQ ID NO: 9 - DNA, 280 bp, synthetic construct
  source 1..280: mol_type = other DNA
ggcagaaaaacctcgacgacaaaactattgccagcttccagcagcagctgtcggatatgggctacaagttccagttcatcaccctggcaggtatccacagcatgtggttcaacatgtttgacctggcaaacgcctatgcctagggcgagggtatgaagcactacgttgagaaagtgcagcagccggaatttgccgccgcgaaagatggctataccttcgtatctcaccagcaggaagtgggtacaggttacttcgataaagtgacgactattattcaggg

SEQ ID NO: 10 - DNA, 1266 bp, synthetic construct
  source 1..1266: mol_type = other DNA
gatgaagagcacaataaccaggtgctcaacaaagtaaaagcggataaatcgctggaagccaataacggtcacgatggcacatggatcgctcacccaggccttgcggacacggcaatggcggtattcaacgacattctcggctcccgtaaaaatcagcttgaagtgatgcgcgaacaagacgcgccgattactgccgatcagctgctggcaccttgtgatggtgaacgcaccgaagaaggtatgcgcgccaacattcgcgtggctgtgcagtacatcgaagcgtggatctctggcaacggctgtgtgccgatttatggcctgatggaagatgcggcgacggctgaaatttcccgtacctcgatctggcagtggatccatcatcaaaaaacgttgagcaatggcaaaccggtgaccaaagccttgttccgccagatgctgggcgaagagatgaaagtcattgccagcgaactgggcgaagaacgtttctcccaggggcgttttgacgatgccgcacgcttgatggaacagatcaccacttccgatgagttaattgatttcctgaccctgccaggctaccgcctgttagcgtaaaccaccacataactatggagcatctgcacgcaacaacaaccgttgctgactgtaggccggataaggcgttcacgccgcatccggcaatcggtgcacgatgcctgatgcgacgcttgcgcgtcttatcatgcctacagccgttgccgaacgtaggctggataaggcgtttacgccgcatccggcaattctctgctcctgatgagggcgctaaatgccgcgtggcctggaattattgattgctcaaaccattttgcaaggcttcgatgctcagtatggtcgattcctcgaagtgacctccggtgcgcagcagcgtttcgaacaggccgactggcatgctgtccagcaggcgatgaaaaaccgtatccatctttacgatcatcacgttggtctggtcgtggagcaactgcgctgcattactaacggccaaagtacggacgcggcatttttactacgtgttaaagagcattacacccggctgttgccggattacccgcgcttcgagattgcggagagcttttttaactccgtgtactgtcggttatttgaccaccgctcgcttactcccgagcggctttttatctttagctctcagccagagcgccgctttcgtaccattccccgcccgctggcgaaagactttcaccccgatcacggctgggaatctctactgatgcg

SEQ ID NO: 11 - DNA, 23 bp, synthetic construct
  source 1..23: mol_type = other DNA
agcggcggacgctaacctggcgg

SEQ ID NO: 12 - DNA, 23 bp, synthetic construct
  source 1..23: mol_type = other DNA
cctggcggccagcatgtatccgg

SEQ ID NO: 13 - DNA, 57 bp, synthetic construct
  source 1..57: mol_type = other DNA
tagcatgactggtggacagcaaatgggtcgcggatcctcttctgtgatagtcgatcg

SEQ ID NO: 14 - DNA, 39 bp, synthetic construct
  source 1..39: mol_type = other DNA
ctccatagttatgtggtggtcgtgcagctcctcgtcatg

SEQ ID NO: 15 - DNA, 40 bp, synthetic construct
  source 1..40: mol_type = other DNA
ccatgacgaggagctgcacgaccaccacataactatggag

SEQ ID NO: 16 - DNA, 58 bp, synthetic construct
  source 1..58: mol_type = other DNA
cggatctcagtggtggtggtggtggtgctcgagtgcttagaactgcgattcttcagtg

SEQ ID NO: 17 - DNA, 20 bp, synthetic construct
  source 1..20: mol_type = other DNA
taatacgactcactataggg

SEQ ID NO: 18 - DNA, 19 bp, synthetic construct
  source 1..19: mol_type = other DNA
gctagttattgctcagcgg

SEQ ID NO: 19 - DNA, 91 bp, synthetic construct
  source 1..91: mol_type = other DNA
tgacagctagctcagtcctaggtataatactagtagcggcggacgctaacctggcgggttttagagctagaaatagcaagttaaaataagg

SEQ ID NO: 20 - DNA, 91 bp, synthetic construct
  source 1..91: mol_type = other DNA
ccttattttaacttgctatttctagctctaaaacccgccaggttagcgtccgccgctactagtattatacctaggactgagctagctgtca

SEQ ID NO: 21 - DNA, 24 bp, synthetic construct
  source 1..24: mol_type = other DNA
gtctcatgagcggatacatatttg

SEQ ID NO: 22 - DNA, 18 bp, synthetic construct
  source 1..18: mol_type = other DNA
atgagaaagcgccacgct

SEQ ID NO: 23 - DNA, 20 bp, synthetic construct
  source 1..20: mol_type = other DNA
ttggcggtgtcctgaatgcc

SEQ ID NO: 24 - DNA, 36 bp, synthetic construct
  source 1..36: mol_type = other DNA
cataccctcgccctaggcataggcgtttgccaggtc

SEQ ID NO: 25 - DNA, 34 bp, synthetic construct
  source 1..34: mol_type = other DNA
aaacgcctatgcctagggcgagggtatgaagcac

SEQ ID NO: 26 - DNA, 21 bp, synthetic construct
  source 1..21: mol_type = other DNA
gtaaaaatgccgcgtccgtac

SEQ ID NO: 27 - DNA, 20 bp, synthetic construct
  source 1..20: mol_type = other DNA
ggcagaaaaacctcgacgac

SEQ ID NO: 28 - DNA, 20 bp, synthetic construct
  source 1..20: mol_type = other DNA
ccctgaataatagtcgtcac

SEQ ID NO: 29 - DNA, 18 bp, synthetic construct
  source 1..18: mol_type = other DNA
gcagtggcggttttcatg

SEQ ID NO: 30 - DNA, 20 bp, synthetic construct
  source 1..20: mol_type = other DNA
ccttggtgatctcgcctttc

SEQ ID NO: 31 - DNA, 91 bp, synthetic construct
  source 1..91: mol_type = other DNA
tgacagctagctcagtcctaggtataatactagtcctggcggccagcatgtatccgggttttagagctagaaatagcaagttaaaataagg

SEQ ID NO: 32 - DNA, 91 bp, synthetic construct
  source 1..91: mol_type = other DNA
ccttattttaacttgctatttctagctctaaaacccggatacatgctggccgccaggactagtattatacctaggactgagctagctgtca

SEQ ID NO: 33 - DNA, 22 bp, synthetic construct
  source 1..22: mol_type = other DNA
gatgaagagcacaataaccagg

SEQ ID NO: 34 - DNA, 45 bp, synthetic construct
  source 1..45: mol_type = other DNA
cagtcagcaacggttgttgttgcgtgcagatgctccatagttatg

SEQ ID NO: 35 - DNA, 45 bp, synthetic construct
  source 1..45: mol_type = other DNA
cataactatggagcatctgcacgcaacaacaaccgttgctgactg

SEQ ID NO: 36 - DNA, 22 bp, synthetic construct
  source 1..22: mol_type = other DNA
cgcatcagtagagattcccagc